European Patent Application EP 4 202 041 A1, published June 28, 2023. Title: Method for expanding human primordial germ cells/human primordial germ cell-like cells. Applicant: Kyoto University. The sequence listing filed with the application follows.

SEQUENCE LISTING (32 sequences)

SEQ ID NO: 1 - DNA, 23 bp, Artificial Sequence
  Primer
gatcccggaagatacgctctaag

SEQ ID NO: 2 - DNA, 23 bp, Artificial Sequence
  Primer
cgcaggttgatgcttccaataaa

SEQ ID NO: 3 - DNA, 23 bp, Artificial Sequence
  Primer
caggcaagagttcaatcgcttag

SEQ ID NO: 4 - DNA, 23 bp, Artificial Sequence
  Primer
tagccttcagtgactgtgagatg

SEQ ID NO: 5 - DNA, 22 bp, Artificial Sequence
  Primer
ccaaccccacattgtaacttcg

SEQ ID NO: 6 - DNA, 22 bp, Artificial Sequence
  Primer
gtctttacttacgcgctcctct

SEQ ID NO: 7 - DNA, 22 bp, Artificial Sequence
  Primer
gaaactctgcattctcgcttcc

SEQ ID NO: 8 - DNA, 22 bp, Artificial Sequence
  Primer
actcgtttgtacccgttgatga

SEQ ID NO: 9 - DNA, 22 bp, Artificial Sequence
  Primer
ttgatcatttggtgtgttgggc

SEQ ID NO: 10 - DNA, 22 bp, Artificial Sequence
  Primer
aagactgagatgcacaagtggt

SEQ ID NO: 11 - DNA, 20 bp, Artificial Sequence
  Primer
ctgtctccgtcaccactctg

SEQ ID NO: 12 - DNA, 20 bp, Artificial Sequence
  Primer
aaaccctggcacaaactcca

SEQ ID NO: 13 - DNA, 22 bp, Artificial Sequence
  Primer
agaggtctcgtatttgctgcat

SEQ ID NO: 14 - DNA, 22 bp, Artificial Sequence
  Primer
aaacactcggtgaaatcagggt

SEQ ID NO: 15 - DNA, 22 bp, Artificial Sequence
  Primer
tgaatcagtctgccgagaatcc

SEQ ID NO: 16 - DNA, 23 bp, Artificial Sequence
  Primer
tctcaaactgtgcataatggagt

SEQ ID NO: 17 - DNA, 22 bp, Artificial Sequence
  Primer
aaaccaaagcatcacgttgaca

SEQ ID NO: 18 - DNA, 22 bp, Artificial Sequence
  Primer
ggatggatggtgagagaagcaa

SEQ ID NO: 19 - DNA, 22 bp, Artificial Sequence
  Primer
attaagaggatgctgggctctg

SEQ ID NO: 20 - DNA, 22 bp, Artificial Sequence
  Primer
cactgtactgcacactcacctt

SEQ ID NO: 21 - DNA, 21 bp, Artificial Sequence
  Primer
acacgtcaggatagttgcagt

SEQ ID NO: 22 - DNA, 20 bp, Artificial Sequence
  Primer
ttcgtgtgcaagcctgagat

SEQ ID NO: 23 - DNA, 22 bp, Artificial Sequence
  Primer
aagcccaaagtcagtgagatga

SEQ ID NO: 24 - DNA, 23 bp, Artificial Sequence
  Primer
gctatagcccaactacctaatgc

SEQ ID NO: 25 - DNA, 25 bp, Artificial Sequence
  Primer
tttttgtctttgttggagtgaagca

SEQ ID NO: 26 - DNA, 25 bp, Artificial Sequence
  Primer
acagtatcagcaataggcagaagca

SEQ ID NO: 27 - DNA, 26 bp, Artificial Sequence
  Primer
actgatacaaatggtgttaactggga

SEQ ID NO: 28 - DNA, 25 bp, Artificial Sequence
  Primer
aaacatgtctaagccccctaaagaa

SEQ ID NO: 29 - DNA, 25 bp, Artificial Sequence
  Primer
caaatgttcagtgtgagtgaggaaa

SEQ ID NO: 30 - DNA, 25 bp, Artificial Sequence
  Primer
tctccccaaagatcacattaactcc

SEQ ID NO: 31 - DNA, 25 bp, Artificial Sequence
  Primer
gtttcatttggagtgtgggacatta

SEQ ID NO: 32 - DNA, 25 bp, Artificial Sequence
  Primer
aacgcttccaaggaaaatcagaaaa